European Patent Specification EP 3 039 131 B1, published January 21, 2026. Title: ENZYME COMPOSITION AND USES THEREOF. Applicant: Novozymes Jump, Joseph Akerman, Michael Kreel, Nathaniel Saunders, Jeremy. The sequence listing filed with the application follows.

SEQUENCE LISTING (20 sequences)

SEQ ID NO: 1 - protein, 515 aa, Bacillus stearothermophilus
  mat_peptide (1)..(515)
AAPFNGTMMQYFEWYLPDDGTLWTKVANEANNLSSLGITALWLPPAYKGTSRSDVGYGVYDLYDLGEFNQKGTVRTKYGTKAQYLQAIQAAHAAGMQVYADVVFDHKGGADGTEWVDAVEVNPSDRNQEISGTYQIQAWTKFDFPGRGNTYSSFKWRWYHFDGVDWDESRKLSRIYKFRGIGKAWDWEVDTENGNYDYLMYADLDMDHPEVVTELKNWGKWYVNTTNIDGFRLDAVKHIKFSFFPDWLSYVRSQTGKPLFTVGEYWSYDINKLHNYITKTNGTMSLFDAPLHNKFYTASKSGGAFDMRTLMTNTLMKDQPTLAVTFVDNHDTEPGQALQSWVDPWFKPLAYAFILTRQEGYPCVFYGDYYGIPQYNIPSLKSKIDPLLIARRDYAYGTQHDYLDHSDIIGWTREGVTEKPGSGLAALITDGPGGSKWMYVGKQHAGKVFYDLTGNRSDTVTINSDGWGEFKVNGGSVSVWVPRKTTVSTIARPITTRPWTGEFVRWTEPRLVAWP

SEQ ID NO: 2 - DNA, 1068 bp, Thermoascus aurantiacus
  CDS (1)..(1065)
  misc_signal (1)..(57)
  misc_feature (58)..(534)
  mat_peptide (535)..(1068)
atgcggctcgttgcttccctaacggccttggtggccttgtccgtacctgtctttcccgctgctgtcaacgtgaagcgtgcttcgtcctacctggagatcactctgagccaggtcagcaacactctgatcaaggccgtggtccagaacactggtagcgacgagttgtccttcgttcacctgaacttcttcaaggaccccgctcctgtcaaaaaggtatcggtctatcgcgatgggtctgaagtgcagttcgagggcattttgagccgctacaaatcgactggcctctctcgtgacgcctttacttatctggctcccggagagtccgtcgaggacgtttttgatattgcttcgacttacgatctgaccagcggcggccctgtaactatccgtactgagggagttgttccctacgccacggctaacagcactgatattgccggctacatctcatactcgtctaatgtgttgaccattgatgtcgatggcgccgctgctgccactgtctccaaggcaatcactcctttggaccgccgcactaggatcagttcctgctccggcagcagacagagcgctcttactacggctctcagaaacgctgcttctcttgccaacgcagctgccgacgcggctcagtctggatcagcttcaaagttcagcgagtacttcaagactacttctagctctacccgccagaccgtggctgcgcgtcttcgggctgttgcgcgggaggcatcttcgtcttcttcgggagccaccacgtactactgcgacgatccctacggctactgttcctccaacgtcctggcttacaccctgccttcatacaacataatcgccaactgtgacattttctatacttacctgccggctctgaccagtacctgtcacgctcaggatcaagcgaccactgcccttcacgagttcacccatgcgcctggcgtctacagccctggcacggacgacctggcgtatggctaccaggctgcgatgggtctcagcagcagccaggctgtcatgaacgctgacacctacgctctctatgcgaatgccatataccttggttgctaa

SEQ ID NO: 3 - protein, 355 aa, Thermoascus aurantiacus
MRLVASLTALVALSVPVFPAAVNVKRASSYLEITLSQVSNTLIKAVVQNTGSDELSFVHLNFFKDPAPVKKVSVYRDGSEVQFEGILSRYKSTGLSRDAFTYLAPGESVEDVFDIASTYDLTSGGPVTIRTEGVVPYATANSTDIAGYISYSSNVLTIDVDGAAAATVSKAITPLDRRTRISSCSGSRQSALTTALRNAASLANAAADAAQSGSASKFSEYFKTTSSSTRQTVAARLRAVAREASSSSSGATTYYCDDPYGYCSSNVLAYTLPSYNIIANCDIFYTYLPALTSTCHAQDQATTALHEFTHAPGVYSPGTDDLAYGYQAAMGLSSSQAVMNADTYALYANAIYLGC

SEQ ID NO: 4 - protein, 573 aa, Gloeophyllum sepiarium
MYRFLVCALGLAASVLAQSVDSYVSSEGPIAKAGVLANIGPNGSKASGASAGVVVASPSTSDPDYWYTWTRDSSLVFKSLIDQYTTGIDSTSSLRTLIDDFVTAEANLQQVSNPSGTLTTGGLGEPKFNVDETAFTGAWGRPQRDGPALRSTALITYGNWLLSNGNTSYVTSNLWPIIQNDLGYVVSYWNQSTYDLWEEVDSSSFFTTAVQHRALREGAAFATAIGQTSQVSSYTTQADNLLCFLQSYWNPSGGYITANTGGGRSGKDANTLLASIHTYDPSAGCDAATFQPCSDKALSNLKVYVDSFRSVYSINSGVASNAAVATGRYPEDSYQGGNPWYLTTFAVAEQLYDALNVWESQGSLEVTSTSLAFFQQFSSGVTAGTYSSSSSTYSTLTSAIKNFADGFVAINAKYTPSNGGLAEQYSKSDGSPLSAVDLTWSYASALTAFEARNNTQFAGWGAAGLTVPSSCSGNSGGPTVAVTFNVNAETVWGENIYLTGSVDALENWSADNALLLSSANYPTWSITVNLPASTAIEYKYIRKNNGAVTWESDPNNSITTPASGSTTENDTWR

SEQ ID NO: 5 - protein, 412 aa, Pyrococcus furiosus
  mat_peptide (1)..(412): Pyrococcus furiosus protease (Pfu)
AELEGLDESAAQVMATYVWNLGYDGSGITIGIIDTGIDASHPDLQGKVIGWVDFVNGRSYPYDDHGHGTHVASIAAGTGAASNGKYKGMAPGAKLAGIKVLGADGSGSISTIIKGVEWAVDNKDKYGIKVINLSLGSSQSSDGTDALSQAVNAAWDAGLVVVVAAGNSGPNKYTIGSPAAASKVITVGAVDKYDVITSFSSRGPTADGRLKPEVVAPGNWIIAARASGTSMGQPINDYYTAAPGTSMATPHVAGIAALLLQAHPSWTPDKVKTALIETADIVKPDEIADIAYGAGRVNAYKAINYDNYAKLVFTGYVANKGSQTHQFVISGASFVTATLYWDNANSDLDLYLYDPNGNQVDYSYTAYYGFEKVGYYNPTDGTWTIKVVSYSGSANYQVDVVSDGSLSQPGSS

SEQ ID NO: 6 - protein, 532 aa, Aspergillus fumigatus
MLASTFSYRMYKTALILAALLGSGQAQQVGTSQAEVHPSMTWQSCTAGGSCTTNNGKVVIDANWRWVHKVGDYTNCYTGNTWDTTICPDDATCASNCALEGANYESTYGVTASGNSLRLNFVTTSQQKNIGSRLYMMKDDSTYEMFKLLNQEFTFDVDVSNLPCGLNGALYFVAMDADGGMSKYPTNKAGAKYGTGYCDSQCPRDLKFINGQANVEGWQPSSNDANAGTGNHGSCCAEMDIWEANSISTAFTPHPCDTPGQVMCTGDACGGTYSSDRYGGTCDPDGCDFNSFRQGNKTFYGPGMTVDTKSKFTVVTQFITDDGTSSGTLKEIKRFYVQNGKVIPNSESTWTGVSGNSITTEYCTAQKSLFQDQNVFEKHGGLEGMGAALAQGMVLVMSLWDDHSANMLWLDSNYPTTASSTTPGVARGTCDISSGVPADVEANHPDAYVVYSNIKVGPIGSTFNSGGSNPGGGTTTTTTTQPTTTTTTAGNPGGTGVAQHYGQCGGIGWTGPTTCASPYTCQKLNDYYSQCL

SEQ ID NO: 7 - protein, 454 aa, Aspergillus fumigatus
MKHLASSIALTLLLPAVQAQQTVWGQCGGQGWSGPTSCVAGAACSTLNPYYAQCIPGATATSTTLTTTTAATTTSQTTTKPTTTGPTTSAPTVTASGNPFSGYQLYANPYYSSEVHTLAMPSLPSSLQPKASAVAEVPSFVWLDVAAKVPTMGTYLADIQAKNKAGANPPIAGIFVVYDLPDRDCAALASNGEYSIANNGVANYKAYIDAIRAQLVKYSDVHTILVIEPDSLANLVTNLNVAKCANAQSAYLECVDYALKQLNLPNVAMYLDAGHAGWLGWPANLGPAATLFAKVYTDAGSPAAVRGLATNVANYNAWSLSTCPSYTQGDPNCDEKKYINAMAPLLKEAGFDAHFIMDTSRNGVQPTKQNAWGDWCNVIGTGFGVRPSTNTGDPLQDAFVWIKPGGESDGTSNSTSPRYDAHCGYSDALQPAPEAGTWFQAYFEQLLTNANPSF

SEQ ID NO: 8 - protein, 863 aa, Aspergillus fumigatus
MRFGWLEVAALTAASVANAQELAFSPPFYPSPWADGQGEWADAHRRAVEIVSQMTLAEKVNLTTGTGWEMDRCVGQTGSVPRLGINWGLCGQDSPLGIRFSDLNSAFPAGTNVAATWDKTLAYLRGKAMGEEFNDKGVDILLGPAAGPLGKYPDGGRIWEGFSPDPVLTGVLFAETIKGIQDAGVIATAKHYILNEQEHFRQVGEAQGYGYNITETISSNVDDKTMHELYLWPFADAVRAGVGAVMCSYNQINNSYGCQNSQTLNKLLKAELGFQGFVMSDWSAHHSGVGAALAGLDMSMPGDISFDDGLSFWGTNLTVSVLNGTVPAWRVDDMAVRIMTAYYKVGRDRLRIPPNFSSWTRDEYGWEHSAVSEGAWTKVNDFVNVQRSHSQIIREIGAASTVLLKNTGALPLTGKEVKVGVLGEDAGSNPWGANGCPDRGCDNGTLAMAWGSGTANFPYLVTPEQAIQREVISNGGNVFAVTDNGALSQMADVASQSSVSLVFVNADSGEGFISVDGNEGDRKNLTLWKNGEAVIDTVVSHCNNTIVVIHSVGPVLIDRWYDNPNVTAIIWAGLPGQESGNSLVDVLYGRVNPSAKTPFTWGKTRESYGAPLLTEPNNGNGAPQDDFNEGVFIDYRHFDKRNETPIYEFGHGLSYTTFGYSHLRVQALNSSSSAYVPTSGETKPAPTYGEIGSAADYLYPEGLKRITKFIYPWLNSTDLEDSSDDPNYGWEDSEYIPEGARDGSPQPLLKAGGAPGGNPTLYQDLVRVSATITNTGNVAGYEVPQLYVSLGGPNEPRVVLRKFDRIFLAPGEQKVWTTTLNRRDLANWDVEAQDWVITKYPKKVHVGSSSRKLPLRAPLPRVY

SEQ ID NO: 9 - protein, 250 aa, Thermoascus aurantiacus
  SIGNAL (1)..(22)
MSFSKIIATAGVLASASLVAGHGFVQNIVIDGKKYYGGYLVNQYPYMSNPPEVIAWSTTATDLGFVDGTGYQTPDIICHRGAKPGALTAPVSPGGTVELQWTPWPDSHHGPVINYLAPCNGDCSTVDKTQLEFFKIAESGLINDDNPPGIWASDNLIAANNSWTVTIPTTIAPGNYVLRHEIIALHSAQNQDGAQNYPQCINLQVTGGGSDNPAGTLGTALYHDTDPGILINIYQKLSSYIIPGPPLYTG

SEQ ID NO: 10 - protein, 253 aa, Penicillium emersonii
  SIGNAL (1)..(25)
MLSSTTRTLAFTGLAGLLSAPLVKAHGFVQGIVIGDQFYSGYIVNSFPYESNPPPVIGWATTATDLGFVDGTGYQGPDIICHRNATPAPLTAPVAAGGTVELQWTPWPDSHHGPVITYLAPCNGNCSTVDKTTLEFFKIDQQGLIDDTSPPGTWASDNLIANNNSWTVTIPNSVAPGNYVLRHEIIALHSANNKDGAQNYPQCINIEVTGGGSDAPEGTLGEDLYHDTDPGILVDIYEPIATYTIPGPPEPTF

SEQ ID NO: 11 - protein, 618 aa, Talaromyces emersonii
MASLVAGALCILGLTPAAFARAPVAARATGSLDSFLATETPIALQGVLNNIGPNGADVAGASAGIVVASPSRSDPNYFYSWTRDAALTAKYLVDAFIAGNKDLEQTIQQYISAQAKVQTISNPSGDLSTGGLGEPKFNVNETAFTGPWGRPQRDGPALRATALIAYANYLIDNGEASTADEIIWPIVQNDLSYITQYWNSSTFDLWEEVEGSSFFTTAVQHRALVEGNALATRLNHTCSNCVSQAPQVLCFLQSYWTGSYVLANFGGSGRSGKDVNSILGSIHTFDPAGGCDDSTFQPCSARALANHKVVTDSFRSIYAINSGIAEGSAVAVGRYPEDVYQGGNPWYLATAAAAEQLYDAIYQWKKIGSISITDVSLPFFQDIYPSAAVGTYNSGSTTFNDIISAVQTYGDGYLSIVEKYTPSDGSLTEQFSRTDGTPLSASALTWSYASLLTASARRQSVVPASWGESSASSVPAVCSATSATGPYSTATNTVWPSSGSGSSTTTSSAPCTTPTSVAVTFDEIVSTSYGETIYLAGSIPELGNWSTASAIPLRADAYTNSNPLWYVTVNLPPGTSFEYKFFKNQTDGTIVWEDDPNRSYTVPAYCGQTTAILDDSWQ

SEQ ID NO: 12 - protein, 574 aa, Trametes cingulata
MRFTLLTSLLGLALGAFAQSSAADAYVASESPIAKAGVLANIGPSGSKSNGAKAGIVIASPSTSNPNYLYTWTRDSSLVFKALIDQFTTGEDTSLRTLIDEFTSAEAILQQVPNPSGTVSTGGLGEPKFNIDETAFTDAWGRPQRDGPALRATAIITYANWLLDNKNTTYVTNTLWPIIKLDLDYVASNWNQSTFDLWEEINSSSFFTTAVQHRALREGATFANRIGQTSVVSGYTTQANNLLCFLQSYWNPTGGYITANTGGGRSGKDANTVLTSIHTFDPAAGCDAVTFQPCSDKALSNLKVYVDAFRSIYSINSGIASNAAVATGRYPEDSYMGGNPWYLTTSAVAEQLYDALIVWNKLGALNVTSTSLPFFQQFSSGVTVGTYASSSSTFKTLTSAIKTFADGFLAVNAKYTPSNGGLAEQYSRSNGSPVSAVDLTWSYAAALTSFAARSGKTYASWGAAGLTVPTTCSGSGGAGTVAVTFNVQATTVFGENIYITGSVPALQNWSPDNALILSAANYPTWSITVNLPASTTIEYKYIRKFNGAVTWESDPNNSITTPASGTFTQNDTWR

SEQ ID NO: 13 - protein, 583 aa, Rhizomucor pusillus
ATSDDWKGKAIYQLLTDRFGRADDSTSNCSNLSNYCGGTYEGITKHLDYISGMGFDAIWISPIPKNSDGGYHGYWATDFYQLNSNFGDESQLKALIQAAHERDMYVMLDVVANHAGPTSNGYSGYTFGDASLYHPKCTIDYNDQTSIEQCWVADELPDIDTENSDNVAILNDIVSGWVGNYSFDGIRIDTVKHIRKDFWTGYAEAAGVFATGEVFNGDPAYVGPYQKYLPSLINYPMYYALNDVFVSKSKGFSRISEMLGSNRNAFEDTSVLTTFVDNHDNPRFLNSQSDKALFKNALTYVLLGEGIPIVYYGSEQGFSGGADPANREVLWTTNYDTSSDLYQFIKTVNSVRMKSNKAVYMDIYVGDNAYAFKHGDALVVLNNYGSGSTNQVSFSVSGKFDSGASLMDIVSNITTTVSSDGTVTFNLKDGLPAIFTSATGGTTTTATPTGSGSVTSTSKTTATASKTSTSTSSTSCTTPTAVAVTFDLTATTTYGENIYLVGSISQLGDWETSDGIALSADKYTSSDPLWYVTVTLPAGESFEYKFIRIESDDSVEWESDPNREYTVPQACGTSTATVTDTWR

SEQ ID NO: 14 - protein, 661 aa, Trichoderma reesei
LYINGSVIAPCDSPIYCHGDILREIELAHPFSDSKTFVDMPAKRPLSEIQTAFANLPKPLRNDSSLQTFLASYFADAGGELIQVPRANLTTNPTFLSKINDTVIEQFVTQVIDIWPDLTRRYAGDAAVKNCSSCPNSFIPVNRTFVVAGGRFREPYYWDSYWIVEGLLRTGGAFVGIARNTIDNFLDFIERFGFVPNGARLYYLNRSQPPLLSRMVKVYIDHTNDTAILRRALPLLVKEHEFWTRNRTVDVRVNNKTYVLNQYAVQNTQPRPESFREDFQTANNRSYYAASGIIYPATKPLNESQIEELYANLASGAESGNDYTARWLADPSDAMRDVYFPLRSLNNKDIVPVDLNSILYGNELAIAQFYNQTGNTTAAREWSSLAANRSASIQAVFWNETLFSYFDYNLTSSSQNIYVPLDKDAVALDRQTAPPGKQVLFHVGQFYPFWTGAAPEYLRNNPFAVTRIFDRVKSYLDTRPGGIPASNVNTGQQWDQPNVWPPHMHILMESLNSVPATFSEADPAYQDVRNLSLRLGQRYLDFTFCTWRATGGSTSETPKLQGLTDQDVGIMFEKYNDNSTNAAGGGGEYQVVEGFGWTNGVLLWTADTFGSQLKRPQCGNIMAGHPAPSKRSAVQLDMWDASRVKKFGRRAEGRMGTLHAW

SEQ ID NO: 15 - protein, 862 aa, Bacillus sp.
  SIGNAL (1)..(33)
MSLIRSRYNHFVILFTVAIMFLTVCFPAYKALADSTSTEVIVHYHRFDSNYANWDLWMWPYQPVNGNGAAYEFSGKDDFGVKADVQVPGDDTQVGLIVRTNDWSQKNTSDDLHIDLTKGHEIWIVQGDPNIYYNLSDAQAAATPKVSNAYLDNEKTVLAKLTNPMTLSDGSSGFTVTDKTTGEQIPVTAATNANSASSSEQTDLVQLTLASAPDVSHTIQVGAAGYEAVNLIPRNVLNLPRYYYSGNDLGNVYSNKATAFRVWAPTASDVQLLLYNSETGPVTKQLEMQKSDNGTWKLKVPGNLKNWYYLYQVTVNGKTQTAVDPYVRAISVNATRGMIVDLEDTNPPGWKEDHQQTPANPVDEVIYEVHVRDFSIDANSGMKNKGKYLAFTEHGTKGPDNVKTGIDSLKELGINAVQLQPIEEFNSIDETQPNMYNWGYDPRNYNVPEGAYATTPEGTARITQLKQLIQSIHKDRIAINMDVVYNHTFNVGVSDFDKIVPQYYYRTDSAGNYTNGSGVGNEIATERPMVQKFVLDSVKYWVKEYHIDGFRFDLMALLGKDTMAKISKELHAINPGIVLYGEPWTGGTSGLSSDQLVTKGQQKGLGIGVFNDNIRNGLDGNVFDKSAQGFATGDPNQVNVIKNGVMGSISDFTSAPSETINYVTSHDNMTLWDKISASNPNDTQADRIKMDELAQAVVFTSQGVPFMQGGEEMLRTKGGNDNSYNAGDSVNQFDWSRKAQFENVFDYYSWLIHLRDNHPAFRMTTADQIKQNLTFLDSPTNTVAFELKNHANHDKWKNIIVMYNPNKTAQTLTLPSGNWTIVGLGNQVGEKSLGHVNGTVEVPALSTIILHQGTSEDVIDQN

SEQ ID NO: 16 - protein, 616 aa, Penicillium oxalicum
MRLTLLSGVAGVLCAGQLTAARPDPKGGNLTPFIHKEGERSLQGILDNLGGRGKKTPGTAAGLFIASPNTENPNYYYTWTRDSALTAKCLIDLFEDSRAKFPIDRKYLETGIRDYVSSQAILQSVSNPSGTLKDGSGLGEPKFEIDLNPFSGAWGRPQRDGPALRATAMITYANYLISHGQKSDVSQVMWPIIANDLAYVGQYWNNTGFDLWEEVDGSSFFTIAVQHRALVEGSQLAKKLGKSCDACDSQPPQILCFLQSFWNGKYITSNINTQASRSGIDLDSVLGSIHTFDPEAACDDATFQPCSARALANHKVYVDSFRSIYKINAGLAEGSAANVGRYPEDVYQGGNPWYLATLGASELLYDALYQWDRLGKLEVSETSLSFFKDFDATVKIGSYSRNSKTYKKLTQSIKSYADGFIQLVQQYTPSNGSLAEQYDRNTAAPLSANDLTWSFASFLTATQRRDAVVPPSWGAKSANKVPTTCSASPVVGTYKAPTATFSSKTKCVPAKDIVPITFYLIENTYYGENVFMSGNITALGNWDAKKGFPLTANLYTQDQNLWFASVEFIPAGTPFEYKYYKVEPNGDITWEKGPNRVFVAPTGCPVQPHSNDVWQF

SEQ ID NO: 17 - protein, 573 aa, Pycnoporus sanguineus
  SIGNAL (1)..(18)
MRFTLLASLIGLAVGAFAQSSAVDAYVASESPIAKQGVLNNIGPNGSKAHGAKAGIVVASPSTENPDYLYTWTRDSSLVFKLLIDQFTSGDDTSLRGLIDDFTSAEAILQQVSNPSGTVSTGGLGEPKFNIDETAFTGAWGRPQRDGPALRATSIIRYANWLLDNGNTTYVSNTLWPVIQLDLDYVADNWNQSTFDLWEEVDSSSFFTTAVQHRALREGATFASRIGQSSVVSGYTTQADNLLCFLQSYWNPSGGYVTANTGGGRSGKDSNTVLTSIHTFDPAAGCDAATFQPCSDKALSNLKVYVDAFRSIYTINNGIASNAAVATGRYPEDSYMGGNPWYLTTSAVAEQLYDALYVWDQLGGLNVTSTSLAFFQQFASGLSTGTYSASSSTYATLTSAIRSFADGFLAINAKYTPADGGLAEQYSRNDGTPLSAVDLTWSYAAALTAFAAREGKTYGSWGAAGLTVPASCSGGGGATVAVTFNVQATTVFGENIYITGSVAALQNWSPDNALILSAANYPTWSITVNLPANTVVQYKYIRKFNGQVTWESDPNNQITTPSGGSFTQNDVWR

SEQ ID NO: 18 - protein, 576 aa, Gloephyllum trabeum
  SIGNAL (1)..(17)
  mat_peptide (18)..(576)
MYRFLVCALGLLGTVLAQSVDSYVGSEGPIAKAGVLANIGPNGSKASGAAAGVVVASPSKSDPDYWYTWTRDSSLVFKSLIDQYTTGIDSTSSLRSLIDSFVIAEANIQQVSNPSGTLTTGGLGEPKFNVDETAFTGAWGRPQRDGPALRATALITYGNWLLSNGNTTWVTSTLWPIIQNDLNYVVQYWNQTTFDLWEEVNSSSFFTTAVQHRALREGAAFATKIGQTSSVSSYTTQAANLLCFLQSYWNPTSGYITANTGGGRSGKDANTLLASIHTYDPSAGCDATTFQPCSDKALSNLKVYVDSFRSVYSINSGIASNAAVATGRYPEDSYQGGNPWYLTTFAVAEQLYDALNVWAAQGSLNVTSISLPFFQQFSSSVTAGTYASSSTTYTTLTSAIKSFADGFVAINAQYTPSNGGLAEQFSRSNGAPVSAVDLTWSYASALTAFEARNNTQFAGWGAVGLTVPTSCSSNSGGGGGSTVAVTFNVNAQTVWGENIYITGSVDALSNWSPDNALLLSSANYPTWSITVNLPASTAIQYKYIRKNNGAVTWESDPNNSITTPASGSVTENDTWR

SEQ ID NO: 19 - protein, 366 aa, Meripilus giganteus [sequence omitted]

SEQ ID NO: 20 - protein, 371 aa, Meripilus giganteus
AIPASCASTITPACLQAIYGIPTTKATQSSNKLAVSGFIDQFANKADLKSFLAQFRKDISSSTTFSLQTLDGGENDQSPSEAGIEANLDIQYTVGLATGVPTTFISVGDDFQDGNLEGFLDIINFLLGESNPPQVLTTSYGQNENTISAKLANQLCNAYAQLGARGTSILFASGDGGVSGSQSAHCSNFVPTFPSGCPFMTSVGATQGVSPETAAAFSSGGFSNVFGIPSYQASAVSGYLSALGSTNSGKFNRSGRGFPDVSTQGVDFQIVSGGQTIGVDGTSCASPTFASVISLVNDRLIAAGKSPLGFLNPFLYSSAGKAALNDVTSGSNPGCSTNGFPAKAGWDPVTGLGTPNFAKLLTAVGLRHQHQ